European Patent Application EP 4 230 734 A1, published August 23, 2023. Title: TYPE II CRISPR/CAS9 GENOME EDITING SYSTEM AND THE APPLICATION THEREOF. Applicant: ZHUHAI SHU TONG MEDICAL TECHNOLOGY CO., LID. The sequence listing filed with the application follows.

SEQUENCE LISTING (33 sequences)

SEQ ID NO: 1 - protein, 1372 aa, Faecalibaculum rodentium
MCTKESEKLNKNADYYIGLDMGTSSAGWAVSDSEYNLIRRKGKDLWGVRQFEEAKTAAERRGFRVARRRKQRQQVRNRLLSEEFQNEITKIDSGFLKRMEDSRFVISDKRVPEKYTLFNDSGYTDVEYYNQYPTIYHLRKALIESNERFDIRLVFLGIHSLFQHPGHFLDKGDVDTDNTGPEELIQFLEDCMNEIQISIPLVSNQKVLTDILTDSRITRRDKEQQILEILQPNKESKKAVSQFVKVLTGQKAKLGDLIMMEDKDTEEYKYSFSFREKTLEEILPDIEGVIDGLALEYIESIYSLYSWSLLNSYMKDTLTGHYYSYLAEARVAAYDKHHSDLVKLKTLFREYIPEEYDNFFRKMEKANYSHYIGSTEYDGEKRCRTAKAKQEDFYKSINKMLEKIPECSEKTEIQKEIIEGTFLLKQTGPQNGFVPNQLQLKELRKILQNASKHYPFLTEKDERDMTAIDRIEALFSFRIPYYIGPLKNTDNQGHGWAVRRDGHEQIPVRPWNFEEIIDESASADLFIKNLVNSCTYLRTEKVLPKSSLLYQEFEVLNELNNLRINGMYPDEIQPGLKRMIFEQCFYSGKKVTGKKLQLFLRSVLTNSSTEEFVLTGIDKDFKSSLSSYKKFCELFGVKTLNDTQKVMAEQIIEWSTVYGDSRKFLKRKLEDNYPELTDQQIRRIAGFKFSEWGNLSRAFLEMEGYKDEAGNPVTIIRALRDTQKNLMQLLSNDSAFAKKLQELNDYVTRDIWSIEPDDLDGMYLSAPVRRMIWQTFLILREVVDTIGYSPKKIFMEMARGEQEKKRTASRKKQLIDLYKEAGMKNDELFGDLESLEEAQLRSKKLYLYFRQMGRDIYSGKLIDFMDVLHGNRYDIDHIHPQSKKKDDSLENNLVLTSKDFNNHIKQDVYPIPEQIQSRQKGFWAMLLKQGFMSQEKYNRLMRTTPFTDEELAEFVNRQLVETRQGTKAIISLINQCFPDSEVVYVKAGNTSDFRQRFDIPKSRDLNNYHHAVDAYLNIVVGNVYDTKFTKNPINFIKKMRKSGNLHSYSLRRMYDFNVQRGDQTAWVAENDTTLKTVKKTAFKTSPMVTKRTYERKGGLADSVLIAAKKAKPGVHLPVKTSDSRFANQVSTYGGYDNVKGSHFFLVEHQQKKKTIRSIENVPIHLKEKLKTKEELEHYCAQVLGMVQPDVRLTRIPMYSLLLIDGYYYYLTGRTGGNLSLSNAVELCLPAKEQAHIRMISKIAGGRSTDALSAEAKDDFRKKNLRLYDELAEKHRSTIFSKRKNPIGPKLLKYREAFVKQTIENQCKVILQILKLTSTNCKTSADLKLIGGSGQEGVMSISKLLRAEKYAEFYLICQSPSGIYETRKNLLTI

SEQ ID NO: 2 - protein, 294 aa, Faecalibaculum rodentium
MTWRTITISSHSKLDYQMGYLVVRGESIKRIHLSEISVLIIENTAVSLTAYLVSELVKNKIKLLFCDEKRSPLAEVSELYGGHDSSDMVRKQIEIPQERKDIAWQSIIMSKISNQFAVLHNFDCPNQELLLQYINEVLPGDVTNREGHAAKVYFNSLFGKSFYRASECALNAALNYGYSVLLSAVSREIAGYGFLTQLGIFHDNCDNKYNLSCDLMEPFRPVVDYLVKSNIVEVFEKEQKQKILQLLQFKIQINDRQETVQNAISIFVHSVLDYLLDPSVYIKVPRIDFTKNVV

SEQ ID NO: 3 - protein, 68 aa, Faecalibaculum rodentium
MMQESVYCKLTTNQSSAETVLKMVRANKPPEGLIQTLIITEKQFSKMDFILGQPNSDVVATDESVLDL

SEQ ID NO: 4 - protein, 223 aa, Faecalibaculum rodentium
MRLLIDRLLLSAELNIDKATTIIIENPKAFRMVIKDLIEQENGQGGLLRIVEGDKELCLSKSAILVLNPYLADLNCRKFLQLAYSELQAMTGEFLEDQAVVLSAMTGYLSKICDQSRFDFLEFSAIPDWASVFKAWGLRFEQAIPGLLPSLIQYLQLAATFPQFKLIIFINLKQYLLPEEQFELFKMAEYLQLKVLLVESAQNYKSDREDLIIIDKDLCEIQS

SEQ ID NO: 5 - RNA, 20 nt, Faecalibaculum rodentium
guuugagugucuuguuaauu

SEQ ID NO: 6 - DNA, 36 bp, Faecalibaculum rodentium
gtttgagtgtcttgttaattcggaagtatttcaaac

SEQ ID NO: 7 - DNA, 216 bp, Faecalibaculum rodentium
gtttgagtgtcttgttaattcgggagtagctctctcgtttgagtgtcttgttaattcggaagtaagctcaacttttgagtgtcttgttaattcggaagtatctcaaacgtttgagtgtcttgttaattcagaagtatttcaaacgtttgagtgtcttgttaattcggaagtattccaaacgtttgagtgtcttgttaattcggaagtatttcaaac

SEQ ID NO: 8 - RNA, 71 nt, Faecalibaculum rodentium
aauuaacaagaugaguucaaaucaggcuccuagagagauccgaacuuaccuucauggcgggcauugugccc

SEQ ID NO: 9 - RNA, 95 nt, Faecalibaculum rodentium
guuugagugucuuguuaauugaaaaauuaacaagaugaguucaaaucaggcuccuagagagauccgaacuuaccuucauggcgggcauugugccc

SEQ ID NO: 10 - RNA, 91 nt, Faecalibaculum rodentium
guuugagugucuuguuaagaaauuaacaagaugaguucaaaucaggcuccuagagagauccgaacuuaccuucauggcgggcauugugccc

SEQ ID NO: 11 - RNA, 89 nt, Faecalibaculum rodentium
guuugagugucuuguuagaaauaacaagaugaguucaaaucaggcuccuagagagauccgaacuuaccuucauggcgggcauugugccc

SEQ ID NO: 12 - RNA, 87 nt, Faecalibaculum rodentium
guuugagugucuuguugaaaaacaagaugaguucaaaucaggcuccuagagagauccgaacuuaccuucauggcgggcauugugccc

SEQ ID NO: 13 - RNA, 85 nt, Faecalibaculum rodentium
guuugagugucuugugaaaacaagaugaguucaaaucaggcuccuagagagauccgaacuuaccuucauggcgggcauugugccc

SEQ ID NO: 14 - RNA, 83 nt, Faecalibaculum rodentium
guuugagugucuuggaaacaagaugaguucaaaucaggcuccuagagagauccgaacuuaccuucauggcgggcauugugccc

SEQ ID NO: 15 - RNA, 79 nt, Faecalibaculum rodentium
guuugagugucugaaaagaugaguucaaaucaggcuccuagagagauccgaacuuaccuucauggcgggcauugugccc

SEQ ID NO: 16 - RNA, 75 nt, Faecalibaculum rodentium
guuugagugugaaaaugaguucaaaucaggcuccuagagagauccgaacuuaccuucauggcgggcauugugccc

SEQ ID NO: 17 - RNA, 71 nt, Faecalibaculum rodentium
guuugagugaaagaguucaaaucaggcuccuagagagauccgaacuuaccuucauggcgggcauugugccc

SEQ ID NO: 18 - DNA, 69 bp, Artificial Sequence
  Synthetic
ctacctgcataccgttattaacatatgacaactcaattaaacgccacatccatcggcgctttggtcggc

SEQ ID NO: 19 - DNA, 62 bp, Artificial Sequence
  Synthetic
atgttaccactggattgaggataccgttattaacatatgacaactcaattaaactctggtac

SEQ ID NO: 20 - DNA, 69 bp, Artificial Sequence
  Synthetic
tcagtttatatgagttacaacgaacaccgtttaattgagttgtcatatgttaataacggtattcaggta

SEQ ID NO: 21 - DNA, 69 bp, Artificial Sequence
  Synthetic
ctacctacataccgttattaacatatgacaactcaattaaacgtcagcacctgggaccccgccaccgtg

SEQ ID NO: 22 - DNA, 34 bp, Artificial Sequence
  Synthetic
gtttaattgagttgtcatatgttaataacggtat

SEQ ID NO: 23 - DNA, 26 bp, Artificial Sequence
  misc_feature (22)..(26): n is a, c, g, or t;r is a or g;w is a or t
tgttaccactggattgaggtcnnrwr

SEQ ID NO: 24 - DNA, 26 bp, Artificial Sequence
  Synthetic
tgttaccactggattgaggtctggta

SEQ ID NO: 25 - DNA, 26 bp, Artificial Sequence
  Synthetic
aagaaccactggattgaggtctggct

SEQ ID NO: 26 - DNA, 26 bp, Artificial Sequence
  Synthetic
gggaaccactggattaaggtccagat

SEQ ID NO: 27 - DNA, 26 bp, Artificial Sequence
  Synthetic
agttaccaatggattgagatggggag

SEQ ID NO: 28 - DNA, 26 bp, Artificial Sequence
  misc_feature (22)..(26): n is a, c, g, or t;r is a or g;w is a or t
aaaaaggaaggagttctttgtnnrwr

SEQ ID NO: 29 - DNA, 26 bp, Artificial Sequence
  Synthetic
aaaaaggaaggagttctttgtaggta

SEQ ID NO: 30 - DNA, 26 bp, Artificial Sequence
  Synthetic
taaaaggaaggtgttctttgtggggt

SEQ ID NO: 31 - DNA, 26 bp, Artificial Sequence
  Synthetic
gaaaaggaaggtgctctttgtgggtg

SEQ ID NO: 32 - DNA, 26 bp, Artificial Sequence
  Synthetic
ggaaaaggtggaattctttgttggta

SEQ ID NO: 33 - DNA, 17 bp, Artificial Sequence
  Synthetic
cgaacacctcaggtaat